European Patent Application EP 4 779 021 A1, published July 22, 2026. Title: MHC gene cluster deficient animal cells. Applicant: Tokyo Metropolitan Institute of Medical Science. The sequence listing filed with the application follows.

SEQUENCE LISTING (101 sequences)

SEQ ID NO: 1 - DNA, 5327 bp, synthetic construct
  misc_feature 1..5327: note = Synthetic DNA
  misc_feature 30..1217: note = /label="EF1"
  misc_feature 1230..2267: note = /label="Hyg"
  misc_feature 2274..2808: note = /label="RGpA"
  misc_feature 3562..4176: note = complement /label="Origin pMB1 ori (pUC)"
  misc_feature 4336..5196: note = complement /label="Bacterial Selection Amp"
  source 1..5327: mol_type = other DNA
gtcgacattgattattgactagatcatcgcgtgaggctccggtgcccgtcagtgggcagagcgcacatcgcccacagtccccgagaagttggggggaggggtcggcaattgaaccggtgcctagagaaggtggcgcggggtaaactgggaaagtgatgtcgtgtactggctccgcctttttcccgagggtgggggagaaccgtatataagtgcagtagtcgccgtgaacgttctttttcgcaacgggtttgccgccagaacacaggtaagtgccgtgtgtggttcccgcgggcctggcctctttacgggttatggcccttgcgtgccttgaattacttccacgcccctggctgcagtacgtgattcttgatcccgagcttcgggttggaagtgggtgggagagttcgaggccttgcgcttaaggagccccttcgcctcgtgcttgagttgaggcctggcctgggcgctggggccgccgcgtgcgaatctggtggcaccttcgcgcctgtctcgctgctttcgataagtctctagccatttaaaatttttgatgacctgctgcgacgctttttttctggcaagatagtcttgtaaatgcgggccaagatctgcacactggtatttcggtttttggggccgcgggcggcgacggggcccgtgcgtcccagcgcacatgttcggcgaggcggggcctgcgagcgcggccaccgagaatcggacgggggtagtctcaagctggccggcctgctctggtgcctggcctcgcgccgccgtgtatcgccccgccctgggcggcaaggctggcccggtcggcaccagttgcgtgagcggaaagatggccgcttcccggccctgctgcagggagctcaaaatggaggacgcggcgctcgggagagcgggcgggtgagtcacccacacaaaggaaaagggcctttccgtcctcagccgtcgcttcatgtgactccacggagtaccgggcgccgtccaggcacctcgattagttctcgagcttttggagtacgtcgtctttaggttggggggaggggttttatgcgatggagtttccccacactgagtgggtggagactgaagttaggccagcttggcacttgatgtaattctccttggaatttgccctttttgagtttggatcttggttcattctcaagcctcagacagtggttcaaagtttttttcttccatttcaggtgtcgtgaggaattgccaccatgaagaagcccgaactcaccgctaccagcgttgaaaaatttctcatcgagaagttcgacagtgtgagcgacctgatgcagttgtcggagggcgaagagagccgagccttcagcttcgatgtcggcggacgcggctatgtactgcgggtgaatagctgcgctgatggcttctacaaagaccgctacgtgtaccgccacttcgccagcgctgcactacccatccccgaagtgttggacatcggcgagttcagcgagagcctgacatactgcatcagtagacgcgcccaaggcgttactctccaagacctccccgaaacagagctgcctgctgtgttacagcctgtcgccgaagctatggatgctattgccgccgccgacctcagtcaaaccagcggcttcggcccattcgggccccaaggcatcggccagtacacaacctggcgggatttcatttgcgccattgctgatccccatgtctaccactggcagaccgtgatggacgacaccgtgtccgccagcgtagctcaagccctggacgaactgatgctgtgggccgaagactgtcccgaggtgcgccacctcgtccatgccgacttcggcagcaacaacgtcctgaccgacaacggccgcatcaccgccgtaatcgactggtccgaagctatgttcggggacagtcagtacgaggtggccaacatcttcttctggcggccctggctggcttgcatggagcagcagactcgctacttcgagcgccggcatcccgagctggccggcagccctcgtctgcgagcctacatgctgcgcatcggcctggatcagctctaccagagcctcgtggacggcaacttcgacgatgctgcctgggctcaaggccgctgcgatgccatcgtccgcagcggggccggcaccgtcggtcgcacacaaatcgctcgccggagcgcagccgtatggaccgacggctgcgtcgaggtgctggccgacagcggcaaccgccggcccagtacacgaccgcgcgctaaggaggtaggtcgagtttaaggccgcactcctcaggtgcaggctgcctatcagaaggtggtggctggtgtggccaatgccctggctcacaaataccactgagatctttttccctctgccaaaaattatggggacatcatgaagccccttgagcatctgacttctggctaataaaggaaatttattttcattgcaatagtgtgttggaattttttgtgtctctcactcggaaggacatatgggagggcaaatcatttaaaacatcagaatgagtatttggtttagagtttggcaacatatgccatatgctggctgccatgaacaaaggtggctataaagaggtcatcagtatatgaaacagccccctgctgtccattccttattccatagaaaagccttgacttgaggttagattttttttatattttgttttgtgttatttttttctttaacatccctaaaattttccttacatgttttactagccagatttttcctcctctcctgactactcccagtcatagctgtccctcttctcttatgaagatccctcgacctgcagcccaagcttggcgtaatcatggtcatagctgtttcctgtgtgaaattgttatccgctcacaattccacacaacatacgagccggaagcataaagtgtaaagcctggggtgcctaatgagtgagctaactcacattaattgcgttgcgctcactgcccgctttccagtcgggaaacctgtcgtgccagcggatccgcatctcaattagtcagcaaccatagtcccgcccctaactccgcccatcccgcccctaactccgcccagttccgcccattctccgccccatggctgactaattttttttatttatgcagaggccgaggccgcctcggcctctgagctattccagaagtagtgaggaggcttttttggaggcctaggcttttgcaaaaagctaacttgtttattgcagcttataatggttacaaataaagcaatagcatcacaaatttcacaaataaagcatttttttcactgcattctagttgtggtttgtccaaactcatcaatgtatcttatcatgtctggatccgctgcattaatgaatcggccaacgcgcggggagaggcggtttgcgtattgggcgctcttccgcttcctcgctcactgactcgctgcgctcggtcgttcggctgcggcgagcggtatcagctcactcaaaggcggtaatacggttatccacagaatcaggggataacgcaggaaagaacatgtgagcaaaaggccagcaaaaggccaggaaccgtaaaaaggccgcgttgctggcgtttttccataggctccgcccccctgacgagcatcacaaaaatcgacgctcaagtcagaggtggcgaaacccgacaggactataaagataccaggcgtttccccctggaagctccctcgtgcgctctcctgttccgaccctgccgcttaccggatacctgtccgcctttctcccttcgggaagcgtggcgctttctcaatgctcacgctgtaggtatctcagttcggtgtaggtcgttcgctccaagctgggctgtgtgcacgaaccccccgttcagcccgaccgctgcgccttatccggtaactatcgtcttgagtccaacccggtaagacacgacttatcgccactggcagcagccactggtaacaggattagcagagcgaggtatgtaggcggtgctacagagttcttgaagtggtggcctaactacggctacactagaaggacagtatttggtatctgcgctctgctgaagccagttaccttcggaaaaagagttggtagctcttgatccggcaaacaaaccaccgctggtagcggtggtttttttgtttgcaagcagcagattacgcgcagaaaaaaaggatctcaagaagatcctttgatcttttctacggggtctgacgctcagtggaacgaaaactcacgttaagggattttggtcatgagattatcaaaaaggatcttcacctagatccttttaaattaaaaatgaagttttaaatcaatctaaagtatatatgagtaaacttggtctgacagttaccaatgcttaatcagtgaggcacctatctcagcgatctgtctatttcgttcatccatagttgcctgactccccgtcgtgtagataactacgatacgggagggcttaccatctggccccagtgctgcaatgataccgcgagacccacgctcaccggctccagatttatcagcaataaaccagccagccggaagggccgagcgcagaagtggtcctgcaactttatccgcctccatccagtctattaattgttgccgggaagctagagtaagtagttcgccagttaatagtttgcgcaacgttgttgccattgctacaggcatcgtggtgtcacgctcgtcgtttggtatggcttcattcagctccggttcccaacgatcaaggcgagttacatgatcccccatgttgtgcaaaaaagcggttagctccttcggtcctccgatcgttgtcagaagtaagttggccgcagtgttatcactcatggttatggcagcactgcataattctcttactgtcatgccatccgtaagatgcttttctgtgactggtgagtactcaaccaagtcattctgagaatagtgtatgcggcgaccgagttgctcttgcccggcgtcaatacgggataataccgcgccacatagcagaactttaaaagtgctcatcattggaaaacgttcttcggggcgaaaactctcaaggatcttaccgctgttgagatccagttcgatgtaacccactcgtgcacccaactgatcttcagcatcttttactttcaccagcgtttctgggtgagcaaaaacaggaaggcaaaatgccgcaaaaaagggaataagggcgacacggaaatgttgaatactcatactcttcctttttcaatattattgaagcatttatcagggttattgtctcatgagcggatacatatttgaatgtatttagaaaaataaacaaataggggttccgcgcacatttccccgaaaagtgccacctg

SEQ ID NO: 2 - DNA, 927 bp, synthetic construct
  misc_feature 1..927: note = Synthetic DNA
  misc_feature 18..65: note = /label="FRT"
  misc_feature 66..342: note = complement /label="BGHpA"
  misc_feature 347..805: note = complement /label="3'Neo"
  misc_feature 806..871: note = /label="SA"
  misc_feature 872..905: note = complement /label="loxP"
  source 1..927: mol_type = other DNA
agtgccacctggtcgacgaagttcctattccgaagttcctattctctagaaagtataggaacttcccccagctggttctttccgcctcagaagccatagagcccaccgcatccccagcatgcctgctattgtcttcccaatcctcccccttgctgtcctgccccaccccaccccccagaatagaatgacacctactcagacaatgcgatgcaatttcctcattttattaggaaaggacagtgggagtggcaccttccagggtcaaggaaggcacgggggaggggcaaacaacagatggctggcaactagaaggcacagtcgaggctgatcagcgagctctaggaattcagaagaactcgtccagcagtctgtagaaggcgatccgctggctgtcaggggcggcaattccatacagcaccaggaaccggtcggcccactctccgcccagttcttcggcaatgtcccgggtggccagggcgatatcctggtatctgtcggccacgcccagtctgccgcagtcgataaagccgctgaaccggccgttttccaccatgatgttgggcaggcaggcatccccgtgtgtcacgaccagatcgtcgccgtcgggcattctggccttcagtctagcaaacagctcggcgggagccagtccctggtgttcttcatccaggtcgtcctggtccaccaggccggcttccattctggttctggcccgctcgatccggtgcttggcttgatgatcgaatggacaggtggcaggatccagggtgtgcagtctccgcatggcgtcggccatgatggacacctgtggagagaaaggcaaagtggatgtcagtaagaccaataggtgcctatcagaaacgcaagagtcataacttcgtataatgtatgctatacgaagttatgaattcgacattgattattgac

SEQ ID NO: 3 - DNA, 25 bp, synthetic construct
  misc_feature 1..25: note = Synthetic DNA
  source 1..25: mol_type = other DNA
aattagccatgtgtggtggcacacg

SEQ ID NO: 4 - DNA, 25 bp, synthetic construct
  misc_feature 1..25: note = Synthetic DNA
  source 1..25: mol_type = other DNA
ccctgagagtcctgtgcatatcagc

SEQ ID NO: 5 - DNA, 20 bp, synthetic construct
  misc_feature 1..20: note = Synthetic DNA
  source 1..20: mol_type = other DNA
tgaggcaggagaatcacttg

SEQ ID NO: 6 - DNA, 27 bp, synthetic construct
  misc_feature 1..27: note = Synthetic DNA
  source 1..27: mol_type = other DNA
gctaaggattaaatcactgcggttatc

SEQ ID NO: 7 - DNA, 39 bp, synthetic construct
  misc_feature 1..39: note = Synthetic DNA
  source 1..39: mol_type = other DNA
gacctgcagcccaagctaccagggataacaggggaacag

SEQ ID NO: 8 - DNA, 38 bp, synthetic construct
  misc_feature 1..38: note = Synthetic DNA
  source 1..38: mol_type = other DNA
gaataggaacttcgtcgactgtcaagcagctagcaggc

SEQ ID NO: 9 - DNA, 864 bp, synthetic construct
  misc_feature 1..864: note = Synthetic DNA
  misc_feature 46..111: note = /lebel="P2A" /note="P2A"
  misc_feature 118..831: note = /lebel="mRuby2"
  source 1..864: mol_type = other DNA
actactcccagtcatagctggcgcgctaaggaggtaggtcgagttggaagcggagctactaacttcagcctgctgaagcaggctggagacgtggaggagaaccctggaccttacgtaatggtgtccaagggcgaggaactgatcaaagaaaacatgcggatgaaggtcgtgatggaaggcagcgtgaacggccaccagttcaagtgtacaggcgagggcgagggcaacccctacatgggcacccagaccatgcggatcaaagtgatcgagggcggacccctgcccttcgcctttgatatcctggccaccagctttatgtacggcagcagaaccttcatcaagtaccccaagggcatccccgatttcttcaagcagagcttccccgagggcttcacctgggagagagtgaccagatacgaggacggcggcgtcgtgaccgtgatgcaggataccagcctggaagatggctgcctggtgtaccacgtgcaagtgcggggcgtgaacttccccagcaacggccctgtgatgcagaaaaagaccaagggctgggagcccaacaccgagatgatgtaccctgccgacggcggcctgagaggctacacacacatggccctgaaggtggacggcggaggccacctgagctgtagcttcgtgaccacctaccggtccaagaaaaccgtgggcaacatcaagatgcccggcatccacgccgtggaccaccggctggaaagactggaagagtccgacaacgagatgttcgtggtgcagcgcgagcatgccgtggccaagtttgctggactgggcggaggcatggacgagctgtacaaatgaggtaccgcgcgcggaggattgggaagacaatag

SEQ ID NO: 10 - DNA, 20 bp, synthetic construct
  misc_feature 1..20: note = Synthetic DNA
  source 1..20: mol_type = other DNA
actactcccagtcatagctg

SEQ ID NO: 11 - DNA, 21 bp, synthetic construct
  misc_feature 1..21: note = Synthetic DNA
  source 1..21: mol_type = other DNA
ctattgtcttcccaatcctcc

SEQ ID NO: 12 - DNA, 5009 bp, synthetic construct
  misc_feature 1..5009: note = Synthetic DNA
  misc_feature 30..1217: note = /label="EF1"
  misc_feature 1230..1949: note = /label="EGFP"
  misc_feature 1956..2490: note = /label="RGpA"
  misc_feature 3244..3858: note = complement /label="Origin pMB1 ori (pUC)"
  misc_feature 4018..4878: note = /label="Bacterial Selection Amp"
  source 1..5009: mol_type = other DNA
gtcgacattgattattgactagatcatcgcgtgaggctccggtgcccgtcagtgggcagagcgcacatcgcccacagtccccgagaagttggggggaggggtcggcaattgaaccggtgcctagagaaggtggcgcggggtaaactgggaaagtgatgtcgtgtactggctccgcctttttcccgagggtgggggagaaccgtatataagtgcagtagtcgccgtgaacgttctttttcgcaacgggtttgccgccagaacacaggtaagtgccgtgtgtggttcccgcgggcctggcctctttacgggttatggcccttgcgtgccttgaattacttccacgcccctggctgcagtacgtgattcttgatcccgagcttcgggttggaagtgggtgggagagttcgaggccttgcgcttaaggagccccttcgcctcgtgcttgagttgaggcctggcctgggcgctggggccgccgcgtgcgaatctggtggcaccttcgcgcctgtctcgctgctttcgataagtctctagccatttaaaatttttgatgacctgctgcgacgctttttttctggcaagatagtcttgtaaatgcgggccaagatctgcacactggtatttcggtttttggggccgcgggcggcgacggggcccgtgcgtcccagcgcacatgttcggcgaggcggggcctgcgagcgcggccaccgagaatcggacgggggtagtctcaagctggccggcctgctctggtgcctggcctcgcgccgccgtgtatcgccccgccctgggcggcaaggctggcccggtcggcaccagttgcgtgagcggaaagatggccgcttcccggccctgctgcagggagctcaaaatggaggacgcggcgctcgggagagcgggcgggtgagtcacccacacaaaggaaaagggcctttccgtcctcagccgtcgcttcatgtgactccacggagtaccgggcgccgtccaggcacctcgattagttctcgagcttttggagtacgtcgtctttaggttggggggaggggttttatgcgatggagtttccccacactgagtgggtggagactgaagttaggccagcttggcacttgatgtaattctccttggaatttgccctttttgagtttggatcttggttcattctcaagcctcagacagtggttcaaagtttttttcttccatttcaggtgtcgtgaggaattgccaccatggtgagcaagggcgaggagctgttcaccggggtggtgcccatcctggtcgagctggacggcgacgtaaacggccacaagttcagcgtgtccggcgagggcgagggcgatgccacctacggcaagctgaccctgaagttcatctgcaccaccggcaagctgcccgtgccctggcccaccctcgtgaccaccctgacctacggcgtgcagtgcttcagccgctaccccgaccacatgaagcagcacgacttcttcaagtccgccatgcccgaaggctacgtccaggagcgcaccatcttcttcaaggacgacggcaactacaagacccgcgccgaggtgaagttcgagggcgacaccctggtgaaccgcatcgagctgaagggcatcgacttcaaggaggacggcaacatcctggggcacaagctggagtacaactacaacagccacaacgtctatatcatggccgacaagcagaagaacggcatcaaggtgaacttcaagatccgccacaacatcgaggacggcagcgtgcagctcgccgaccactaccagcagaacacccccatcggcgacggccccgtgctgctgcccgacaaccactacctgagcacccagtccgccctgagcaaagaccccaacgagaagcgcgatcacatggtcctgctggagttcgtgaccgccgccgggatcactctcggcatggacgagctgtacaagtaaggccgcactcctcaggtgcaggctgcctatcagaaggtggtggctggtgtggccaatgccctggctcacaaataccactgagatctttttccctctgccaaaaattatggggacatcatgaagccccttgagcatctgacttctggctaataaaggaaatttattttcattgcaatagtgtgttggaattttttgtgtctctcactcggaaggacatatgggagggcaaatcatttaaaacatcagaatgagtatttggtttagagtttggcaacatatgccatatgctggctgccatgaacaaaggtggctataaagaggtcatcagtatatgaaacagccccctgctgtccattccttattccatagaaaagccttgacttgaggttagattttttttatattttgttttgtgttatttttttctttaacatccctaaaattttccttacatgttttactagccagatttttcctcctctcctgactactcccagtcatagctgtccctcttctcttatgaagatccctcgacctgcagcccaagcttggcgtaatcatggtcatagctgtttcctgtgtgaaattgttatccgctcacaattccacacaacatacgagccggaagcataaagtgtaaagcctggggtgcctaatgagtgagctaactcacattaattgcgttgcgctcactgcccgctttccagtcgggaaacctgtcgtgccagcggatccgcatctcaattagtcagcaaccatagtcccgcccctaactccgcccatcccgcccctaactccgcccagttccgcccattctccgccccatggctgactaattttttttatttatgcagaggccgaggccgcctcggcctctgagctattccagaagtagtgaggaggcttttttggaggcctaggcttttgcaaaaagctaacttgtttattgcagcttataatggttacaaataaagcaatagcatcacaaatttcacaaataaagcatttttttcactgcattctagttgtggtttgtccaaactcatcaatgtatcttatcatgtctggatccgctgcattaatgaatcggccaacgcgcggggagaggcggtttgcgtattgggcgctcttccgcttcctcgctcactgactcgctgcgctcggtcgttcggctgcggcgagcggtatcagctcactcaaaggcggtaatacggttatccacagaatcaggggataacgcaggaaagaacatgtgagcaaaaggccagcaaaaggccaggaaccgtaaaaaggccgcgttgctggcgtttttccataggctccgcccccctgacgagcatcacaaaaatcgacgctcaagtcagaggtggcgaaacccgacaggactataaagataccaggcgtttccccctggaagctccctcgtgcgctctcctgttccgaccctgccgcttaccggatacctgtccgcctttctcccttcgggaagcgtggcgctttctcaatgctcacgctgtaggtatctcagttcggtgtaggtcgttcgctccaagctgggctgtgtgcacgaaccccccgttcagcccgaccgctgcgccttatccggtaactatcgtcttgagtccaacccggtaagacacgacttatcgccactggcagcagccactggtaacaggattagcagagcgaggtatgtaggcggtgctacagagttcttgaagtggtggcctaactacggctacactagaaggacagtatttggtatctgcgctctgctgaagccagttaccttcggaaaaagagttggtagctcttgatccggcaaacaaaccaccgctggtagcggtggtttttttgtttgcaagcagcagattacgcgcagaaaaaaaggatctcaagaagatcctttgatcttttctacggggtctgacgctcagtggaacgaaaactcacgttaagggattttggtcatgagattatcaaaaaggatcttcacctagatccttttaaattaaaaatgaagttttaaatcaatctaaagtatatatgagtaaacttggtctgacagttaccaatgcttaatcagtgaggcacctatctcagcgatctgtctatttcgttcatccatagttgcctgactccccgtcgtgtagataactacgatacgggagggcttaccatctggccccagtgctgcaatgataccgcgagacccacgctcaccggctccagatttatcagcaataaaccagccagccggaagggccgagcgcagaagtggtcctgcaactttatccgcctccatccagtctattaattgttgccgggaagctagagtaagtagttcgccagttaatagtttgcgcaacgttgttgccattgctacaggcatcgtggtgtcacgctcgtcgtttggtatggcttcattcagctccggttcccaacgatcaaggcgagttacatgatcccccatgttgtgcaaaaaagcggttagctccttcggtcctccgatcgttgtcagaagtaagttggccgcagtgttatcactcatggttatggcagcactgcataattctcttactgtcatgccatccgtaagatgcttttctgtgactggtgagtactcaaccaagtcattctgagaatagtgtatgcggcgaccgagttgctcttgcccggcgtcaatacgggataataccgcgccacatagcagaactttaaaagtgctcatcattggaaaacgttcttcggggcgaaaactctcaaggatcttaccgctgttgagatccagttcgatgtaacccactcgtgcacccaactgatcttcagcatcttttactttcaccagcgtttctgggtgagcaaaaacaggaaggcaaaatgccgcaaaaaagggaataagggcgacacggaaatgttgaatactcatactcttcctttttcaatattattgaagcatttatcagggttattgtctcatgagcggatacatatttgaatgtatttagaaaaataaacaaataggggttccgcgcacatttccccgaaaagtgccacctg

SEQ ID NO: 13 - DNA, 1285 bp, synthetic construct
  misc_feature 1..1285: note = Synthetic DNA
  misc_feature 22..618: note = complement /label="Puro"
  misc_feature 619..681: note = complement /label="T2A"
  misc_feature 684..750: note = /label="SA"
  misc_feature 751..784: note = complement /label="loxP"
  misc_feature 788..854: note = /label="SD"
  misc_feature 855..1199: note = complement /label="5'Neo"
  misc_feature 1200..1265: note = complement /label="P2A"
  source 1..1285: mol_type = other DNA
tgcggccttacttgtacgaattcaggcgccaggctttctggtcatgcaccaggtggctctatccttggggcattccacgtcggcggtcacggtgaagcccagtctctcgtagaagggcaggtttctgggggcgcttgtttccaggaaggcgggcacgccagccctttcagcagcttccacgccaggcagcaccacagcagatcccagtcccttgccctggtggtcaggtgacacgcccacggtggccagaaaccaggcaggctctttaggtctgtggggggccagcaggccttccatctgctgctgggcagccagtctagagccgctcagctcggccattctaggtccgatctcggcgaacacagcgccggcttccacagactcaggggttgtccacacagccacagcggcgccatcatcggccacccacactttgccgatgtccaggcccactctggtcagaaacagttcctgcagctcggtcactctctcgatgtgtctgtcggggtccacggtgtgtctggtggcagggtaatcggcgaaggcagcggccagtgtccgcacagctctaggcacatcgtccctggtggccagccgcactgtgggcttgtactcggtaggtccaggattctcctccacgtcaccgcatgttagcagacttcctctgccctctccgcttcctacctgtggagagaaaggcaaagtggatgtcagtaagaccaataggtgcctatcagaaacgcaagagtcataacttcgtataatgtatgctatacgaagttatgaattctctgtctcgacaagcccagtttctattggtctccttaaacctgtcttgtaaccttgatacttaccttctcggcaggggccagatggctagacagcagatcctggcctggcacttcgcccagcagcagccagtctcttccggcctctgtcacgacgtccagcacagcggcacatggcacgcctgttgtggccagccagctcagtctggcggcttcatcctgcagctcgttcagggcgccagacaggtcggttttcacgaacagcacgggtctgccctgggcactcagtctgaacacggcggcatcggaacagccgatggtctgctgggcccaatcgtagccgaacagtctttccacccaggcggctggagatccggcgtgcagtccatcctgctcgatggcagagcccataggtccagggttctcctccacgtctccagcctgcttcagcaggctgaagttagtagctccgcttcccttgtacagctcgtccatgc

SEQ ID NO: 14 - DNA, 54 bp, synthetic construct
  misc_feature 1..54: note = Synthetic DNA
  source 1..54: mol_type = other DNA
tcgaggaagttcctattccgaagttcctattctctagaaagtataggaacttcg

SEQ ID NO: 15 - DNA, 54 bp, synthetic construct
  misc_feature 1..54: note = Synthetic DNA
  source 1..54: mol_type = other DNA
tcgacgaagttcctatactttctagagaataggaacttcggaataggaacttcc

SEQ ID NO: 16 - DNA, 26 bp, synthetic construct
  misc_feature 1..26: note = Synthetic DNA
  source 1..26: mol_type = other DNA
gcgtcagatctcattatggatggctg

SEQ ID NO: 17 - DNA, 26 bp, synthetic construct
  misc_feature 1..26: note = Synthetic DNA
  source 1..26: mol_type = other DNA
cgagcctatgagggtcattctcactc

SEQ ID NO: 18 - DNA, 20 bp, synthetic construct
  misc_feature 1..20: note = Synthetic DNA
  source 1..20: mol_type = other DNA
gaactcaggaccttcagaag

SEQ ID NO: 19 - DNA, 25 bp, synthetic construct
  misc_feature 1..25: note = Synthetic DNA
  source 1..25: mol_type = other DNA
caactaacacagttactcccataac

SEQ ID NO: 20 - DNA, 43 bp, synthetic construct
  misc_feature 1..43: note = Synthetic DNA
  source 1..43: mol_type = other DNA
gtataggaacttcgtcgaacgctggtaacatttgccaacatct

SEQ ID NO: 21 - DNA, 44 bp, synthetic construct
  misc_feature 1..44: note = Synthetic DNA
  source 1..44: mol_type = other DNA
acctgcagcccaagctttgttggcctgatatctcattaaatctg

SEQ ID NO: 22 - DNA, 8424 bp, synthetic construct
  misc_feature 1..8424: note = Synthetic DNA
  misc_feature 819..1679: note = /label="Amp"
  misc_feature 1839..2453: note = /label="Origin pMB1 ori (pUC)"
  misc_feature 2957..4041: note = /label="LA"
  misc_feature 4047..5746: note = /label="CAG promoter"
  misc_feature 5756..6412: note = /label="Hprt"
  misc_feature 6439..6968: note = /label="RGpA"
  misc_feature 6975..8363: note = /label="RA"
  source 1..8424: mol_type = other DNA
tatagtgagtcgtattacaattcactggccgtcgttttacaacgtcgtgactgggaaaaccctggcgttacccaacttaatcgccttgcagcacatccccctttcgccagctggcgtaatagcgaagaggcccgcaccgatcgcccttcccaacagttgcgcagcctgaatggcgaatggacgcgccctgtagcggcgcattaagcgcggcgggtgtggtggttacgcgcagcgtgaccgctacacttgccagcgccctagcgcccgctcctttcgctttcttcccttcctttctcgccacgttcgccggctttccccgtcaagctctaaatcgggggctccctttagggttccgatttagtgctttacggcacctcgaccccaaaaaacttgattagggtgatggttcacgtagtgggccatcgccctgatagacggtttttcgccctttgacgttggagtccacgttctttaatagtggactcttgttccaaactggaacaacactcaaccctatctcggtctattcttttgatttataagggattttgccgatttcggcctattggttaaaaaatgagctgatttaacaaaaatttaacgcgaattttaacaaaatattaacgcttacaatttcctgatgcggtattttctccttacgcatctgtgcggtatttcacaccgcatcaggtggcacttttcggggaaatgtgcgcggaacccctatttgtttatttttctaaatacattcaaatatgtatccgctcatgagacaataaccctgataaatgcttcaataatattgaaaaaggaagagtatgagtattcaacatttccgtgtcgcccttattcccttttttgcggcattttgccttcctgtttttgctcacccagaaacgctggtgaaagtaaaagatgctgaagatcagttgggtgcacgagtgggttacatcgaactggatctcaacagcggtaagatccttgagagttttcgccccgaagaacgttttccaatgatgagcacttttaaagttctgctatgtggcgcggtattatcccgtattgacgccgggcaagagcaactcggtcgccgcatacactattctcagaatgacttggttgagtactcaccagtcacagaaaagcatcttacggatggcatgacagtaagagaattatgcagtgctgccataaccatgagtgataacactgcggccaacttacttctgacaacgatcggaggaccgaaggagctaaccgcttttttgcacaacatgggggatcatgtaactcgccttgatcgttgggaaccggagctgaatgaagccataccaaacgacgagcgtgacaccacgatgcctgtagcaatggcaacaacgttgcgcaaactattaactggcgaactacttactctagcttcccggcaacaattaatagactggatggaggcggataaagttgcaggaccacttctgcgctcggcccttccggctggctggtttattgctgataaatctggagccggtgagcgtgggtctcgcggtatcattgcagcactggggccagatggtaagccctcccgtatcgtagttatctacacgacggggagtcaggcaactatggatgaacgaaatagacagatcgctgagataggtgcctcactgattaagcattggtaactgtcagaccaagtttactcatatatactttagattgatttaaaacttcatttttaatttaaaaggatctaggtgaagatcctttttgataatctcatgaccaaaatcccttaacgtgagttttcgttccactgagcgtcagaccccgtagaaaagatcaaaggatcttcttgagatcctttttttctgcgcgtaatctgctgcttgcaaacaaaaaaaccaccgctaccagcggtggtttgtttgccggatcaagagctaccaactctttttccgaaggtaactggcttcagcagagcgcagataccaaatactgttcttctagtgtagccgtagttaggccaccacttcaagaactctgtagcaccgcctacatacctcgctctgctaatcctgttaccagtggctgctgccagtggcgataagtcgtgtcttaccgggttggactcaagacgatagttaccggataaggcgcagcggtcgggctgaacggggggttcgtgcacacagcccagcttggagcgaacgacctacaccgaactgagatacctacagcgtgagctatgagaaagcgccacgcttcccgaagggagaaaggcggacaggtatccggtaagcggcagggtcggaacaggagagcgcacgagggagcttccagggggaaacgcctggtatctttatagtcctgtcgggtttcgccacctctgacttgagcgtcgatttttgtgatgctcgtcaggggggcggagcctatggaaaaacgccagcaacgcggcctttttacggttcctggccttttgctggccttttgctcacatgttctttcctgcgttatcccctgattctgtggataaccgtattaccgcctttgagtgagctgataccgctcgccgcagccgaacgaccgagcgcagcgagtcagtgagcgaggaagcggaagagcgcccaatacgcaaaccgcctctccccgcgcgttggccgattcattaatgcagctggcacgacaggtttcccgactggaaagcgggcagtgagcgcaacgcaattaatgtgagttagctcactcattaggcaccccaggctttacactttatgcttccggctcgtatgttgtgtggaattgtgagcggataacaatttcacacaggaaacagctatgaccatgattacgccaagctatttaggtgacactatagaatactcaagctatgcatccaacgcgttgggagctctcccatatggtcgacctgcaggcggccgcgaattcactagtgattgcctttatgtctctgggtctcatggacaaatagggttaataagagtcctgcaacaaggctgggcgtggtggctcaagcctgtaatcccagcactttgggaggtcgaggtgggcagatcacctgaggtcaggactagcctggccaacacggtgaaacctgtcaccactaaaaatacaaaattagcctggcatagtggcacatgcctgtagtcccagctactggggaggctaaggtgggagaatcacttgaactcgggaggtggaggttgcagtgagccaagatggcaccattgcactccagcctgggcgacaagagtgaaactccatctcaaaaataaataaataaataaaaataaaaatagagtcctgcaacagtgaggatgcattcagatgaaagcaacagaaaactcagctaataatgtcagttaataaagacatttaattgtttcatatttcaaaaatgtccggaggtcagcagccagtaagccccctaacgatattatctaagacccagggtctcttcatcctgctccatcatccttggcgtgctggcttttggggccctctgtgtgatactccactgatattcttggcacatgggaaacatcatctgctcttggatttcccagatcaatctgaggatattacttcttgggggtaggtagggccctgtggtggtttggactgttattcccaatcctttgcttcctccttattatttaagtgtacatccatcccctttgctgtgtgacttgcttgtgccaacagaatgtcagaggacacgatgcaagcagatgctttcaatgtgcttttgtagtttggcttggcctcttgcactcctgtgatctgacaagagaaaggcaaattccagatatccattgccccttcagctgtgacccagaatagacactggaccaggactaaaggagtcctaccaagccctgtcaagcccagcctgattagacaaaccacagacaactcacaaacccatgagcatgaaaataaatagagtggcttaagcaatctcctggggacaggtataggaggacagcaagggtccttgggttctcagagtgtcctccagctggatcctagttattaatagtaatcaattacggggtcattagttcatagcccatatatggagttccgcgttacataacttacggtaaatggcccgcctggctgaccgcccaacgacccccgcccattgacgtcaataatgacgtatgttcccatagtaacgccaatagggactttccattgacgtcaatgggtggactatttacggtaaactgcccacttggcagtacatcaagtgtatcatatgccaagtacgccccctattgacgtcaatgacggtaaatggcccgcctggcattatgcccagtacatgaccttatgggactttcctacttggcagtacatctacgtattagtcatcgctattaccatgggtcgaggtgagccccacgttctgcttcactctccccatctcccccccctccccacccccaattttgtatttatttattttttaattattttgtgcagcgatgggggcggggggggggggggcgcgcgccaggcggggcggggcggggcgaggggcggggcggggcgaggcggagaggtgcggcggcagccaatcagagcggcgcgctccgaaagtttccttttatggcgaggcggcggcggcggcggccctataaaaagcgaagcgcgcggcgggcgggagtcgctgcgttgccttcgccccgtgccccgctccgcgccgcctcgcgccgcccgccccggctctgactgaccgcgttactcccacaggtgagcgggcgggacggcccttctcctccgggctgtaattagcgcttggtttaatgacggctcgtttcttttctgtggctgcgtgaaagccttaaagggctccgggagggccctttgtgcgggggggagcggctcggggggtgcgtgcgtgtgtgtgtgcgtggggagcgccgcgtgcggcccgcgctgcccggcggctgtgagcgctgcgggcgcggcgcggggctttgtgcgctccgcgtgtgcgcgaggggagcgcggccgggggcggtgccccgcggtgcgggggggctgcgaggggaacaaaggctgcgtgcggggtgtgtgcgtgggggggtgagcagggggtgtgggcgcggcggtcgggctgtaacccccccctgcacccccctccccgagttgctgagcacggcccggcttcgggtgcggggctccgtgcggggcgtggcgcggggctcgccgtgccgggcggggggtggcggcaggtgggggtgccgggcggggcggggccgcctcgggccggggagggctcgggggaggggcgcggcggccccggagcgccggcggctgtcgaggcgcggcgagccgcagccattgccttttatggtaatcgtgcgagagggcgcagggacttcctttgtcccaaatctggcggagccgaaatctgggaggcgccgccgcaccccctctagcgggcgcgggcgaagcggtgcggcgccggcaggaaggaaatgggcggggagggccttcgtgcgtcgccgcgccgccgtccccttctccatctccagcctcggggctgccgcagggggacggctgccttcgggggggacggggcagggcggggttcggcttctggcgtgtgaccggcggctctagagcctctgctaaccatgttcatgccttcttctttttcctacagctcctgggcaacgtgctggttattgtgctgtctcatcattttggcaaagaattcaccatgccgacccgcagtcccagcgtcgtgattagcgatgatgaaccaggttatgacctagatttgttttgtatacctaatcattatgccgaggatttggaaaaagtgtttattcctcatggactgattatggacaggactgaaagacttgctcgagatgtcatgaaggagatgggaggccatcacattgtggccctctgtgtgctcaaggggggctataagttctttgctgacctgctggattacattaaagcactgaatagaaatagtgatagatccattcctatgactgtagattttatcagactgaagagctactgtaatgatcagtcaacgggggacataaaagttattggtggagatgatctctcaactttaactggaaagaatgtcttgattgttgaagatataattgacactggtaaaacaatgcaaactttgctttccctggttaagcagtacagccccaaaatggttaaggttgcaagcttgctggtgaaaaggacctctcgaagtgttggatacaggccagactttgttggatttgaaattccagacaagtttgttgttggatatgcccttgactataatgagtacttcagggatttgaatcacgtttgtgtcattagtgaaactggaaaagccaaatacaaagcctaagaattcctcgaggatatcgcggccgcactcctcaggtgcaggctgcctatcagaaggtggtggctggtgtggccaatgccctggctcacaaataccactgagatctttttccctctgccaaaaattatggggacatcatgaagccccttgagcatctgacttctggctaataaaggaaatttattttcattgcaatagtgtgttggaattttttgtgtctctcactcggaaggacatatgggagggcaaatcatttaaaacatcagaatgagtatttggtttagagtttggcaacatatgccatatgctggctgccatgaacaaaggtggctataaagaggtcatcagtatatgaaacagccccctgctgtccattccttattccatagaaaagccttgacttgaggttagattttttttatattttgttttgtgttatttttttctttaacatccctaaaattttccttacatgttttactagccagatttttcctcctctcctgactactcccagtcatagctgtccctcttctcttatgaagatccctcgaccggatccttagggcgagagaaacttcttgactcagtgacatgaattctcttaggagagtcacattagcagctctgttcagttaggagaggccagggccctgggagttcatttgttctctcctgggtgttcagcaccagatgttacttgaggggactcagttaagaaaaggctgacatagcctggcagtggtggcgcatgcctgtaatcccagcacttgggaggcagaggcaggtggatttctgagttcaaggccagcctggtctacagagtgagttccaggaccgacataaggggcaggattgagagatggctcagtggttaagagcactgactgaactttcccttccaggaggggaggggtctggtgtaattttccaaagttcatgagctgacctcttcaacatggctgttatcagggatggtttttagtgtagatatgggggaagggaggggagcgatggcagtctgaggtgagggaggggccaggatgccagggcaggggctctggataacagaacttgtgtgaatagggacagatggcgtctggaggccagcatgggctttgctgggcacccacagatacttgtttatggagagccatttgtcccttctgccagagggaagaaaaatggcttctttttgccagaggggagcaggtttcacaagttctccaggaatgctggtggttgccagaaacccttctctaggccaggttgagtgtgcctgccttttctggaagggcatgtgaggtagatcccacagggatgctatttcaggaggcagaggaaggcagatccctgtcaattcaaggccagcctggactacatgacgagttccaggccagccagggctacaggctgagaccctttctgaaaacctgtacacgaagcagcaagctgcttttttctctaagacagggtttctctgtgtagccctgactggcttggaactcagagatctgcctgcctttgcctctgcctccggcgtcctggaattaaaggcatgtgcaaccacgccagacttctcttttttttttttttttttttttgagacagggtttctctgtgtagtcctggctgtcctggaactcactgtagaccaggctggcctcaaactcagaaatccgcctgcctctgcctcccaagtgctgggattaaaggcatgcaccaccactgcctggctatgccagacttctttgtttatttgaggcaaggtctccatccggtccctcaggctgcccttgaatttggcatggagtggaggatgaccttgaactcacaactcccctgcctcccaatccccagtgttggacagaaggccgacgccacaggtggcttttgaaatgtgaaagattaaatccagggcttcctggaagacaaccacagaattcatggcaatcgaattcccgcggccgccatggcggccgggagcatgcgacgtcgggcccaattcgccc

SEQ ID NO: 23 - DNA, 554 bp, synthetic construct
  misc_feature 1..554: note = Synthetic DNA
  misc_feature 126..524: note = /label="Blasticidin resistance gene"
  source 1..554: mol_type = other DNA
cgtgtgaccggcggctctagagcctctgctaaccatgttcatgccttcttctttttcctacagctcctgggcaacgtgctggttattgtgctgtctcatcattttggcaaagtttaaacgccaccatggccaagcctttgtctcaagaagaatccaccctcattgaaagagcaacggctacaatcaacagcatccccatctctgaagactacagcgtcgccagcgcagctctctctagcgacggccgcatcttcactggtgtcaatgtatatcattttactgggggaccttgtgcagaactcgtggtgctgggcactgctgctgctgcggcagctggcaacctgacttgtatcgtcgcgatcggaaatgagaacaggggcatcttgagcccctgcggacggtgccgacaggtgcttctcgatctgcatcctgggatcaaagccatagtgaaggacagtgatggacagccgacggcagttgggattcgtgaattgctgccctctggttatgtgtgggagggctaatgtttaaacctcgaggatatcgcggccgca

SEQ ID NO: 24 - DNA, 9292 bp, synthetic construct
  misc_feature 1..9292: note = Synthetic DNA
  misc_feature 1..249: note = /label="U6 promoter"
  misc_feature 268..343: note = /label="chimeric guide RNA scaffold"
  misc_feature 344..349: note = /label="U6 terminator"
  misc_feature 440..1238: note = /label="CBh"
  misc_feature 1251..1319: note = /label="3xFLAG"
  misc_feature 1320..1370: note = /label="NLS(1)"
  misc_feature 1371..5471: note = /label="hSpCsn1"
  misc_feature 5472..5519: note = /label="NLS"
  misc_feature 5526..5588: note = /label="T2A"
  misc_feature 5589..6305: note = /label="Ametrine"
  misc_feature 6315..6546: note = /label="BGHpA"
  misc_feature 7612..8472: note = /label="Bacterial Selection Amp"
  misc_feature 8632..9246: note = /label="Origin pMB1 ori (pUC)"
  source 1..9292: mol_type = other DNA
gagggcctatttcccatgattccttcatatttgcatatacgatacaaggctgttagagagataattggaattaatttgactgtaaacacaaagatattagtacaaaatacgtgacgtagaaagtaataatttcttgggtagtttgcagttttaaaattatgttttaaaatggactatcatatgcttaccgtaacttgaaagtatttcgatttcttggctttatatatcttgtggaaaggacgaaacaccgggtcttcgagaagacctgttttagagctagaaatagcaagttaaaataaggctagtccgttatcaacttgaaaaagtggcaccgagtcggtgcttttttgttttagagctagaaatagcaagttaaaataaggctagtccgtttttagcgcgtgcgccaattctgcagacaaatggctctagaggtacccgttacataacttacggtaaatggcccgcctggctgaccgcccaacgacccccgcccattgacgtcaatagtaacgccaatagggactttccattgacgtcaatgggtggagtatttacggtaaactgcccacttggcagtacatcaagtgtatcatatgccaagtacgccccctattgacgtcaatgacggtaaatggcccgcctggcattgtgcccagtacatgaccttatgggactttcctacttggcagtacatctacgtattagtcatcgctattaccatggtcgaggtgagccccacgttctgcttcactctccccatctcccccccctccccacccccaattttgtatttatttattttttaattattttgtgcagcgatgggggcggggggggggggggggcgcgcgccaggcggggcggggcggggcgaggggcggggcggggcgaggcggagaggtgcggcggcagccaatcagagcggcgcgctccgaaagtttccttttatggcgaggcggcggcggcggcggccctataaaaagcgaagcgcgcggcgggcgggagtcgctgcgacgctgccttcgccccgtgccccgctccgccgccgcctcgcgccgcccgccccggctctgactgaccgcgttactcccacaggtgagcgggcgggacggcccttctcctccgggctgtaattagctgagcaagaggtaagggtttaagggatggttggttggtggggtattaatgtttaattacctggagcacctgcctgaaatcactttttttcaggttggaccggtgccaccatggactataaggaccacgacggagactacaaggatcatgatattgattacaaagacgatgacgataagatggccccaaagaagaagcggaaggtcggtatccacggagtcccagcagccgacaagaagtacagcatcggcctggacatcggcaccaactctgtgggctgggccgtgatcaccgacgagtacaaggtgcccagcaagaaattcaaggtgctgggcaacaccgaccggcacagcatcaagaagaacctgatcggagccctgctgttcgacagcggcgaaacagccgaggccacccggctgaagagaaccgccagaagaagatacaccagacggaagaaccggatctgctatctgcaagagatcttcagcaacgagatggccaaggtggacgacagcttcttccacagactggaagagtccttcctggtggaagaggataagaagcacgagcggcaccccatcttcggcaacatcgtggacgaggtggcctaccacgagaagtaccccaccatctaccacctgagaaagaaactggtggacagcaccgacaaggccgacctgcggctgatctatctggccctggcccacatgatcaagttccggggccacttcctgatcgagggcgacctgaaccccgacaacagcgacgtggacaagctgttcatccagctggtgcagacctacaaccagctgttcgaggaaaaccccatcaacgccagcggcgtggacgccaaggccatcctgtctgccagactgagcaagagcagacggctggaaaatctgatcgcccagctgcccggcgagaagaagaatggcctgttcggaaacctgattgccctgagcctgggcctgacccccaacttcaagagcaacttcgacctggccgaggatgccaaactgcagctgagcaaggacacctacgacgacgacctggacaacctgctggcccagatcggcgaccagtacgccgacctgtttctggccgccaagaacctgtccgacgccatcctgctgagcgacatcctgagagtgaacaccgagatcaccaaggcccccctgagcgcctctatgatcaagagatacgacgagcaccaccaggacctgaccctgctgaaagctctcgtgcggcagcagctgcctgagaagtacaaagagattttcttcgaccagagcaagaacggctacgccggctacattgacggcggagccagccaggaagagttctacaagttcatcaagcccatcctggaaaagatggacggcaccgaggaactgctcgtgaagctgaacagagaggacctgctgcggaagcagcggaccttcgacaacggcagcatcccccaccagatccacctgggagagctgcacgccattctgcggcggcaggaagatttttacccattcctgaaggacaaccgggaaaagatcgagaagatcctgaccttccgcatcccctactacgtgggccctctggccaggggaaacagcagattcgcctggatgaccagaaagagcgaggaaaccatcaccccctggaacttcgaggaagtggtggacaagggcgcttccgcccagagcttcatcgagcggatgaccaacttcgataagaacctgcccaacgagaaggtgctgcccaagcacagcctgctgtacgagtacttcaccgtgtataacgagctgaccaaagtgaaatacgtgaccgagggaatgagaaagcccgccttcctgagcggcgagcagaaaaaggccatcgtggacctgctgttcaagaccaaccggaaagtgaccgtgaagcagctgaaagaggactacttcaagaaaatcgagtgcttcgactccgtggaaatctccggcgtggaagatcggttcaacgcctccctgggcacataccacgatctgctgaaaattatcaaggacaaggacttcctggacaatgaggaaaacgaggacattctggaagatatcgtgctgaccctgacactgtttgaggacagagagatgatcgaggaacggctgaaaacctatgcccacctgttcgacgacaaagtgatgaagcagctgaagcggcggagatacaccggctggggcaggctgagccggaagctgatcaacggcatccgggacaagcagtccggcaagacaatcctggatttcctgaagtccgacggcttcgccaacagaaacttcatgcagctgatccacgacgacagcctgacctttaaagaggacatccagaaagcccaggtgtccggccagggcgatagcctgcacgagcacattgccaatctggccggcagccccgccattaagaagggcatcctgcagacagtgaaggtggtggacgagctcgtgaaagtgatgggccggcacaagcccgagaacatcgtgatcgaaatggccagagagaaccagaccacccagaagggacagaagaacagccgcgagagaatgaagcggatcgaagagggcatcaaagagctgggcagccagatcctgaaagaacaccccgtggaaaacacccagctgcagaacgagaagctgtacctgtactacctgcagaatgggcgggatatgtacgtggaccaggaactggacatcaaccggctgtccgactacgatgtggaccatatcgtgcctcagagctttctgaaggacgactccatcgacaacaaggtgctgaccagaagcgacaagaaccggggcaagagcgacaacgtgccctccgaagaggtcgtgaagaagatgaagaactactggcggcagctgctgaacgccaagctgattacccagagaaagttcgacaatctgaccaaggccgagagaggcggcctgagcgaactggataaggccggcttcatcaagagacagctggtggaaacccggcagatcacaaagcacgtggcacagatcctggactcccggatgaacactaagtacgacgagaatgacaagctgatccgggaagtgaaagtgatcaccctgaagtccaagctggtgtccgatttccggaaggatttccagttttacaaagtgcgcgagatcaacaactaccaccacgcccacgacgcctacctgaacgccgtcgtgggaaccgccctgatcaaaaagtaccctaagctggaaagcgagttcgtgtacggcgactacaaggtgtacgacgtgcggaagatgatcgccaagagcgagcaggaaatcggcaaggctaccgccaagtacttcttctacagcaacatcatgaactttttcaagaccgagattaccctggccaacggcgagatccggaagcggcctctgatcgagacaaacggcgaaaccggggagatcgtgtgggataagggccgggattttgccaccgtgcggaaagtgctgagcatgccccaagtgaatatcgtgaaaaagaccgaggtgcagacaggcggcttcagcaaagagtctatcctgcccaagaggaacagcgataagctgatcgccagaaagaaggactgggaccctaagaagtacggcggcttcgacagccccaccgtggcctattctgtgctggtggtggccaaagtggaaaagggcaagtccaagaaactgaagagtgtgaaagagctgctggggatcaccatcatggaaagaagcagcttcgagaagaatcccatcgactttctggaagccaagggctacaaagaagtgaaaaaggacctgatcatcaagctgcctaagtactccctgttcgagctggaaaacggccggaagagaatgctggcctctgccggcgaactgcagaagggaaacgaactggccctgccctccaaatatgtgaacttcctgtacctggccagccactatgagaagctgaagggctcccccgaggataatgagcagaaacagctgtttgtggaacagcacaagcactacctggacgagatcatcgagcagatcagcgagttctccaagagagtgatcctggccgacgctaatctggacaaagtgctgtccgcctacaacaagcaccgggataagcccatcagagagcaggccgagaatatcatccacctgtttaccctgaccaatctgggagcccctgccgccttcaagtactttgacaccaccatcgaccggaagaggtacaccagcaccaaagaggtgctggacgccaccctgatccaccagagcatcaccggcctgtacgagacacggatcgacctgtctcagctgggaggcgacaaaaggccggcggccacgaaaaaggccggccaggcaaaaaagaaaaaggaattcggcagtggagagggcagaggaagtctgctaacatgcggtgacgtcgaggagaatcctggcccagtgagcaagggcgaggagctgttcaccggggtggtgcccatcctggtcgagctggacggcgacgtaaacggccacaggttcagcgtgcgcggcgagggcgagggcgatgccaccaacggcaagctgaccctgaagttcatctgcacctccggcgagctgcccgtgccctggcccaccctcgtgaccaccctgtcttacggcgtgcagtgcttcgcccgctaccccgaccacatgaagcagcacgacttcttcaagtccgccatgcccgaaggctacgtccaggagcgcaccatctccttcaaggacgacggcagctacaggacccgcgccgaggtgaagttcgagggcgacaccctggtgaaccgcatcgagctgaagggcatcgacttcaaggaggacggcaacatcctggggcacaagctggagtacaacatgaacgcgtgggacgcgtatatcacggccgacaagcagaagaacggcatcaaagcgaacttcaagatcgagcacaacgtcaaggacggcggcgtgcagctcgccgacgcgtaccagcagaacacccccatcggcgacggctccgtgctgctgcctgacaaccactacctgagcttccagagcaagctgttcaaagaccccaacgagcagcgcgatcacatggtcctgctggagttcgttaccgccgccgggataactcccggcatggacgagctgtacaagtaagaattctaactagagctcgctgatcagcctcgactgtgccttctagttgccagccatctgttgtttgcccctcccccgtgccttccttgaccctggaaggtgccactcccactgtcctttcctaataaaatgaggaaattgcatcgcattgtctgagtaggtgtcattctattctggggggtggggtggggcaggacagcaagggggaggattgggaagagaatagcaggcatgctggggagcggccgcaggaacccctagtgatggagttggccactccctctctgcgcgctcgctcgctcactgaggccgggcgaccaaaggtcgcccgacgcccgggctttgcccgggcggcctcagtgagcgagcgagcgcgcagctgcctgcaggggcgcctgatgcggtattttctccttacgcatctgtgcggtatttcacaccgcatacgtcaaagcaaccatagtacgcgccctgtagcggcgcattaagcgcggcgggtgtggtggttacgcgcagcgtgaccgctacacttgccagcgccctagcgcccgctcctttcgctttcttcccttcctttctcgccacgttcgccggctttccccgtcaagctctaaatcgggggctccctttagggttccgatttagtgctttacggcacctcgaccccaaaaaacttgatttgggtgatggttcacgtagtgggccatcgccctgatagacggtttttcgccctttgacgttggagtccacgttctttaatagtggactcttgttccaaactggaacaacactcaaccctatctcgggctattcttttgatttataagggattttgccgatttcggcctattggttaaaaaatgagctgatttaacaaaaatttaacgcgaattttaacaaaatattaacgtttacaattttatggtgcactctcagtacaatctgctctgatgccgcatagttaagccagccccgacacccgccaacacccgctgacgcgccctgacgggcttgtctgctcccggcatccgcttacagacaagctgtgaccgtctccgggagctgcatgtgtcagaggttttcaccgtcatcaccgaaacgcgcgagacgaaagggcctcgtgatacgcctatttttataggttaatgtcatgataataatggtttcttagacgtcaggtggcacttttcggggaaatgtgcgcggaacccctatttgtttatttttctaaatacattcaaatatgtatccgctcatgagacaataaccctgataaatgcttcaataatattgaaaaaggaagagtatgagtattcaacatttccgtgtcgcccttattcccttttttgcggcattttgccttcctgtttttgctcacccagaaacgctggtgaaagtaaaagatgctgaagatcagttgggtgcacgagtgggttacatcgaactggatctcaacagcggtaagatccttgagagttttcgccccgaagaacgttttccaatgatgagcacttttaaagttctgctatgtggcgcggtattatcccgtattgacgccgggcaagagcaactcggtcgccgcatacactattctcagaatgacttggttgagtactcaccagtcacagaaaagcatcttacggatggcatgacagtaagagaattatgcagtgctgccataaccatgagtgataacactgcggccaacttacttctgacaacgatcggaggaccgaaggagctaaccgcttttttgcacaacatgggggatcatgtaactcgccttgatcgttgggaaccggagctgaatgaagccataccaaacgacgagcgtgacaccacgatgcctgtagcaatggcaacaacgttgcgcaaactattaactggcgaactacttactctagcttcccggcaacaattaatagactggatggaggcggataaagttgcaggaccacttctgcgctcggcccttccggctggctggtttattgctgataaatctggagccggtgagcgtggaagccgcggtatcattgcagcactggggccagatggtaagccctcccgtatcgtagttatctacacgacggggagtcaggcaactatggatgaacgaaatagacagatcgctgagataggtgcctcactgattaagcattggtaactgtcagaccaagtttactcatatatactttagattgatttaaaacttcatttttaatttaaaaggatctaggtgaagatcctttttgataatctcatgaccaaaatcccttaacgtgagttttcgttccactgagcgtcagaccccgtagaaaagatcaaaggatcttcttgagatcctttttttctgcgcgtaatctgctgcttgcaaacaaaaaaaccaccgctaccagcggtggtttgtttgccggatcaagagctaccaactctttttccgaaggtaactggcttcagcagagcgcagataccaaatactgtccttctagtgtagccgtagttaggccaccacttcaagaactctgtagcaccgcctacatacctcgctctgctaatcctgttaccagtggctgctgccagtggcgataagtcgtgtcttaccgggttggactcaagacgatagttaccggataaggcgcagcggtcgggctgaacggggggttcgtgcacacagcccagcttggagcgaacgacctacaccgaactgagatacctacagcgtgagctatgagaaagcgccacgcttcccgaagggagaaaggcggacaggtatccggtaagcggcagggtcggaacaggagagcgcacgagggagcttccagggggaaacgcctggtatctttatagtcctgtcgggtttcgccacctctgacttgagcgtcgatttttgtgatgctcgtcaggggggcggagcctatggaaaaacgccagcaacgcggcctttttacggttcctggccttttgctggccttttgctcacatgt

SEQ ID NO: 25 - DNA, 20 bp, synthetic construct
  misc_feature 1..20: note = Synthetic DNA
  source 1..20: mol_type = other DNA
ctagctgcttgacagtaacc

SEQ ID NO: 26 - DNA, 20 bp, synthetic construct
  misc_feature 1..20: note = Synthetic DNA
  source 1..20: mol_type = other DNA
gatatcaggccaacaaacgc

SEQ ID NO: 27 - DNA, 9302 bp, synthetic construct
  misc_feature 1..9302: note = Synthetic DNA
  misc_feature 1..249: note = /label="U6 promoter"
  misc_feature 268..353: note = /label="chimeric guide RNA scaffold"
  misc_feature 354..359: note = /label="U6 terminator"
  misc_feature 450..1248: note = /label="CBh"
  misc_feature 1261..1329: note = /label="3xFLAG"
  misc_feature 1330..1380: note = /label="NLS(1)"
  misc_feature 1381..5481: note = /label="hSpCsn1"
  misc_feature 5482..5529: note = /label="NLS"
  misc_feature 5536..5598: note = /label="T2A"
  misc_feature 5599..6315: note = /label="Ametrine"
  misc_feature 6325..6556: note = /label="BGHpA"
  misc_feature 7622..8482: note = /label="Bacterial Selection Amp"
  misc_feature 8642..9256: note = /label="Origine pMB1 ori (pUC)"
  source 1..9302: mol_type = other DNA
gagggcctatttcccatgattccttcatatttgcatatacgatacaaggctgttagagagataattggaattaatttgactgtaaacacaaagatattagtacaaaatacgtgacgtagaaagtaataatttcttgggtagtttgcagttttaaaattatgttttaaaatggactatcatatgcttaccgtaacttgaaagtatttcgatttcttggctttatatatcttgtggaaaggacgaaacaccgggtcttcgagaagacctgtttcagagctatgctggaaacagcatagcaagttgaaataaggctagtccgttatcaacttgaaaaagtggcaccgagtcggtgcttttttgttttagagctagaaatagcaagttaaaataaggctagtccgtttttagcgcgtgcgccaattctgcagacaaatggctctagaggtacccgttacataacttacggtaaatggcccgcctggctgaccgcccaacgacccccgcccattgacgtcaatagtaacgccaatagggactttccattgacgtcaatgggtggagtatttacggtaaactgcccacttggcagtacatcaagtgtatcatatgccaagtacgccccctattgacgtcaatgacggtaaatggcccgcctggcattgtgcccagtacatgaccttatgggactttcctacttggcagtacatctacgtattagtcatcgctattaccatggtcgaggtgagccccacgttctgcttcactctccccatctcccccccctccccacccccaattttgtatttatttattttttaattattttgtgcagcgatgggggcggggggggggggggggcgcgcgccaggcggggcggggcggggcgaggggcggggcggggcgaggcggagaggtgcggcggcagccaatcagagcggcgcgctccgaaagtttccttttatggcgaggcggcggcggcggcggccctataaaaagcgaagcgcgcggcgggcgggagtcgctgcgacgctgccttcgccccgtgccccgctccgccgccgcctcgcgccgcccgccccggctctgactgaccgcgttactcccacaggtgagcgggcgggacggcccttctcctccgggctgtaattagctgagcaagaggtaagggtttaagggatggttggttggtggggtattaatgtttaattacctggagcacctgcctgaaatcactttttttcaggttggaccggtgccaccatggactataaggaccacgacggagactacaaggatcatgatattgattacaaagacgatgacgataagatggccccaaagaagaagcggaaggtcggtatccacggagtcccagcagccgacaagaagtacagcatcggcctggacatcggcaccaactctgtgggctgggccgtgatcaccgacgagtacaaggtgcccagcaagaaattcaaggtgctgggcaacaccgaccggcacagcatcaagaagaacctgatcggagccctgctgttcgacagcggcgaaacagccgaggccacccggctgaagagaaccgccagaagaagatacaccagacggaagaaccggatctgctatctgcaagagatcttcagcaacgagatggccaaggtggacgacagcttcttccacagactggaagagtccttcctggtggaagaggataagaagcacgagcggcaccccatcttcggcaacatcgtggacgaggtggcctaccacgagaagtaccccaccatctaccacctgagaaagaaactggtggacagcaccgacaaggccgacctgcggctgatctatctggccctggcccacatgatcaagttccggggccacttcctgatcgagggcgacctgaaccccgacaacagcgacgtggacaagctgttcatccagctggtgcagacctacaaccagctgttcgaggaaaaccccatcaacgccagcggcgtggacgccaaggccatcctgtctgccagactgagcaagagcagacggctggaaaatctgatcgcccagctgcccggcgagaagaagaatggcctgttcggaaacctgattgccctgagcctgggcctgacccccaacttcaagagcaacttcgacctggccgaggatgccaaactgcagctgagcaaggacacctacgacgacgacctggacaacctgctggcccagatcggcgaccagtacgccgacctgtttctggccgccaagaacctgtccgacgccatcctgctgagcgacatcctgagagtgaacaccgagatcaccaaggcccccctgagcgcctctatgatcaagagatacgacgagcaccaccaggacctgaccctgctgaaagctctcgtgcggcagcagctgcctgagaagtacaaagagattttcttcgaccagagcaagaacggctacgccggctacattgacggcggagccagccaggaagagttctacaagttcatcaagcccatcctggaaaagatggacggcaccgaggaactgctcgtgaagctgaacagagaggacctgctgcggaagcagcggaccttcgacaacggcagcatcccccaccagatccacctgggagagctgcacgccattctgcggcggcaggaagatttttacccattcctgaaggacaaccgggaaaagatcgagaagatcctgaccttccgcatcccctactacgtgggccctctggccaggggaaacagcagattcgcctggatgaccagaaagagcgaggaaaccatcaccccctggaacttcgaggaagtggtggacaagggcgcttccgcccagagcttcatcgagcggatgaccaacttcgataagaacctgcccaacgagaaggtgctgcccaagcacagcctgctgtacgagtacttcaccgtgtataacgagctgaccaaagtgaaatacgtgaccgagggaatgagaaagcccgccttcctgagcggcgagcagaaaaaggccatcgtggacctgctgttcaagaccaaccggaaagtgaccgtgaagcagctgaaagaggactacttcaagaaaatcgagtgcttcgactccgtggaaatctccggcgtggaagatcggttcaacgcctccctgggcacataccacgatctgctgaaaattatcaaggacaaggacttcctggacaatgaggaaaacgaggacattctggaagatatcgtgctgaccctgacactgtttgaggacagagagatgatcgaggaacggctgaaaacctatgcccacctgttcgacgacaaagtgatgaagcagctgaagcggcggagatacaccggctggggcaggctgagccggaagctgatcaacggcatccgggacaagcagtccggcaagacaatcctggatttcctgaagtccgacggcttcgccaacagaaacttcatgcagctgatccacgacgacagcctgacctttaaagaggacatccagaaagcccaggtgtccggccagggcgatagcctgcacgagcacattgccaatctggccggcagccccgccattaagaagggcatcctgcagacagtgaaggtggtggacgagctcgtgaaagtgatgggccggcacaagcccgagaacatcgtgatcgaaatggccagagagaaccagaccacccagaagggacagaagaacagccgcgagagaatgaagcggatcgaagagggcatcaaagagctgggcagccagatcctgaaagaacaccccgtggaaaacacccagctgcagaacgagaagctgtacctgtactacctgcagaatgggcgggatatgtacgtggaccaggaactggacatcaaccggctgtccgactacgatgtggaccatatcgtgcctcagagctttctgaaggacgactccatcgacaacaaggtgctgaccagaagcgacaagaaccggggcaagagcgacaacgtgccctccgaagaggtcgtgaagaagatgaagaactactggcggcagctgctgaacgccaagctgattacccagagaaagttcgacaatctgaccaaggccgagagaggcggcctgagcgaactggataaggccggcttcatcaagagacagctggtggaaacccggcagatcacaaagcacgtggcacagatcctggactcccggatgaacactaagtacgacgagaatgacaagctgatccgggaagtgaaagtgatcaccctgaagtccaagctggtgtccgatttccggaaggatttccagttttacaaagtgcgcgagatcaacaactaccaccacgcccacgacgcctacctgaacgccgtcgtgggaaccgccctgatcaaaaagtaccctaagctggaaagcgagttcgtgtacggcgactacaaggtgtacgacgtgcggaagatgatcgccaagagcgagcaggaaatcggcaaggctaccgccaagtacttcttctacagcaacatcatgaactttttcaagaccgagattaccctggccaacggcgagatccggaagcggcctctgatcgagacaaacggcgaaaccggggagatcgtgtgggataagggccgggattttgccaccgtgcggaaagtgctgagcatgccccaagtgaatatcgtgaaaaagaccgaggtgcagacaggcggcttcagcaaagagtctatcctgcccaagaggaacagcgataagctgatcgccagaaagaaggactgggaccctaagaagtacggcggcttcgacagccccaccgtggcctattctgtgctggtggtggccaaagtggaaaagggcaagtccaagaaactgaagagtgtgaaagagctgctggggatcaccatcatggaaagaagcagcttcgagaagaatcccatcgactttctggaagccaagggctacaaagaagtgaaaaaggacctgatcatcaagctgcctaagtactccctgttcgagctggaaaacggccggaagagaatgctggcctctgccggcgaactgcagaagggaaacgaactggccctgccctccaaatatgtgaacttcctgtacctggccagccactatgagaagctgaagggctcccccgaggataatgagcagaaacagctgtttgtggaacagcacaagcactacctggacgagatcatcgagcagatcagcgagttctccaagagagtgatcctggccgacgctaatctggacaaagtgctgtccgcctacaacaagcaccgggataagcccatcagagagcaggccgagaatatcatccacctgtttaccctgaccaatctgggagcccctgccgccttcaagtactttgacaccaccatcgaccggaagaggtacaccagcaccaaagaggtgctggacgccaccctgatccaccagagcatcaccggcctgtacgagacacggatcgacctgtctcagctgggaggcgacaaaaggccggcggccacgaaaaaggccggccaggcaaaaaagaaaaaggaattcggcagtggagagggcagaggaagtctgctaacatgcggtgacgtcgaggagaatcctggcccagtgagcaagggcgaggagctgttcaccggggtggtgcccatcctggtcgagctggacggcgacgtaaacggccacaggttcagcgtgcgcggcgagggcgagggcgatgccaccaacggcaagctgaccctgaagttcatctgcacctccggcgagctgcccgtgccctggcccaccctcgtgaccaccctgtcttacggcgtgcagtgcttcgcccgctaccccgaccacatgaagcagcacgacttcttcaagtccgccatgcccgaaggctacgtccaggagcgcaccatctccttcaaggacgacggcagctacaggacccgcgccgaggtgaagttcgagggcgacaccctggtgaaccgcatcgagctgaagggcatcgacttcaaggaggacggcaacatcctggggcacaagctggagtacaacatgaacgcgtgggacgcgtatatcacggccgacaagcagaagaacggcatcaaagcgaacttcaagatcgagcacaacgtcaaggacggcggcgtgcagctcgccgacgcgtaccagcagaacacccccatcggcgacggctccgtgctgctgcctgacaaccactacctgagcttccagagcaagctgttcaaagaccccaacgagcagcgcgatcacatggtcctgctggagttcgttaccgccgccgggataactcccggcatggacgagctgtacaagtaagaattctaactagagctcgctgatcagcctcgactgtgccttctagttgccagccatctgttgtttgcccctcccccgtgccttccttgaccctggaaggtgccactcccactgtcctttcctaataaaatgaggaaattgcatcgcattgtctgagtaggtgtcattctattctggggggtggggtggggcaggacagcaagggggaggattgggaagagaatagcaggcatgctggggagcggccgcaggaacccctagtgatggagttggccactccctctctgcgcgctcgctcgctcactgaggccgggcgaccaaaggtcgcccgacgcccgggctttgcccgggcggcctcagtgagcgagcgagcgcgcagctgcctgcaggggcgcctgatgcggtattttctccttacgcatctgtgcggtatttcacaccgcatacgtcaaagcaaccatagtacgcgccctgtagcggcgcattaagcgcggcgggtgtggtggttacgcgcagcgtgaccgctacacttgccagcgccctagcgcccgctcctttcgctttcttcccttcctttctcgccacgttcgccggctttccccgtcaagctctaaatcgggggctccctttagggttccgatttagtgctttacggcacctcgaccccaaaaaacttgatttgggtgatggttcacgtagtgggccatcgccctgatagacggtttttcgccctttgacgttggagtccacgttctttaatagtggactcttgttccaaactggaacaacactcaaccctatctcgggctattcttttgatttataagggattttgccgatttcggcctattggttaaaaaatgagctgatttaacaaaaatttaacgcgaattttaacaaaatattaacgtttacaattttatggtgcactctcagtacaatctgctctgatgccgcatagttaagccagccccgacacccgccaacacccgctgacgcgccctgacgggcttgtctgctcccggcatccgcttacagacaagctgtgaccgtctccgggagctgcatgtgtcagaggttttcaccgtcatcaccgaaacgcgcgagacgaaagggcctcgtgatacgcctatttttataggttaatgtcatgataataatggtttcttagacgtcaggtggcacttttcggggaaatgtgcgcggaacccctatttgtttatttttctaaatacattcaaatatgtatccgctcatgagacaataaccctgataaatgcttcaataatattgaaaaaggaagagtatgagtattcaacatttccgtgtcgcccttattcccttttttgcggcattttgccttcctgtttttgctcacccagaaacgctggtgaaagtaaaagatgctgaagatcagttgggtgcacgagtgggttacatcgaactggatctcaacagcggtaagatccttgagagttttcgccccgaagaacgttttccaatgatgagcacttttaaagttctgctatgtggcgcggtattatcccgtattgacgccgggcaagagcaactcggtcgccgcatacactattctcagaatgacttggttgagtactcaccagtcacagaaaagcatcttacggatggcatgacagtaagagaattatgcagtgctgccataaccatgagtgataacactgcggccaacttacttctgacaacgatcggaggaccgaaggagctaaccgcttttttgcacaacatgggggatcatgtaactcgccttgatcgttgggaaccggagctgaatgaagccataccaaacgacgagcgtgacaccacgatgcctgtagcaatggcaacaacgttgcgcaaactattaactggcgaactacttactctagcttcccggcaacaattaatagactggatggaggcggataaagttgcaggaccacttctgcgctcggcccttccggctggctggtttattgctgataaatctggagccggtgagcgtggaagccgcggtatcattgcagcactggggccagatggtaagccctcccgtatcgtagttatctacacgacggggagtcaggcaactatggatgaacgaaatagacagatcgctgagataggtgcctcactgattaagcattggtaactgtcagaccaagtttactcatatatactttagattgatttaaaacttcatttttaatttaaaaggatctaggtgaagatcctttttgataatctcatgaccaaaatcccttaacgtgagttttcgttccactgagcgtcagaccccgtagaaaagatcaaaggatcttcttgagatcctttttttctgcgcgtaatctgctgcttgcaaacaaaaaaaccaccgctaccagcggtggtttgtttgccggatcaagagctaccaactctttttccgaaggtaactggcttcagcagagcgcagataccaaatactgtccttctagtgtagccgtagttaggccaccacttcaagaactctgtagcaccgcctacatacctcgctctgctaatcctgttaccagtggctgctgccagtggcgataagtcgtgtcttaccgggttggactcaagacgatagttaccggataaggcgcagcggtcgggctgaacggggggttcgtgcacacagcccagcttggagcgaacgacctacaccgaactgagatacctacagcgtgagctatgagaaagcgccacgcttcccgaagggagaaaggcggacaggtatccggtaagcggcagggtcggaacaggagagcgcacgagggagcttccagggggaaacgcctggtatctttatagtcctgtcgggtttcgccacctctgacttgagcgtcgatttttgtgatgctcgtcaggggggcggagcctatggaaaaacgccagcaacgcggcctttttacggttcctggccttttgctggccttttgctcacatgt

SEQ ID NO: 28 - DNA, 20 bp, synthetic construct
  misc_feature 1..20: note = Synthetic DNA
  source 1..20: mol_type = other DNA
gactcataaaccggaggagc

SEQ ID NO: 29 - DNA, 20 bp, synthetic construct
  misc_feature 1..20: note = Synthetic DNA
  source 1..20: mol_type = other DNA
cgtgtagtaggcgcccgtta

SEQ ID NO: 30 - DNA, 26 bp, synthetic construct
  misc_feature 1..26: note = Synthetic DNA
  source 1..26: mol_type = other DNA
agtaaatcctgactgagcacctcctg

SEQ ID NO: 31 - DNA, 22 bp, synthetic construct
  misc_feature 1..22: note = Synthetic DNA
  source 1..22: mol_type = other DNA
gcttgcgtgaggctgaagtgtc

SEQ ID NO: 32 - DNA, 418 bp, synthetic construct
  misc_feature 1..418: note = Synthetic DNA
  source 1..418: mol_type = other DNA
aaggagtttctgagattgcttctgtctagcttttatggaaagatatttccttttctaccataggcctcaaagcgctcttagtatacacttccaaattctacaaagagagtgttactaaaccgctctctcaaaggaaatgttaaactctatgagttgaaacacagcacacaaacagttctgagacacttctgtctgccttttatgtgaagacatccctttccaaagaatgcctccaagggttcaaaatatccacttgtagactttacaaagagagtgttcaaaactttctctaccaaaagaaaggttaaagacggtgagttcaaacgcacacatcacaaagttgtttctaagaatcatctactatgttctagagatgttcctttctatcatagctcaatgtctaaatatccactgaatc

SEQ ID NO: 33 - DNA, 27 bp, synthetic construct
  misc_feature 1..27: note = Synthetic DNA
  source 1..27: mol_type = other DNA
cttggggtccagagaagaaaatcactc

SEQ ID NO: 34 - DNA, 27 bp, synthetic construct
  misc_feature 1..27: note = Synthetic DNA
  source 1..27: mol_type = other DNA
ctctatggcttctgaggcggaaagaac

SEQ ID NO: 35 - DNA, 22 bp, synthetic construct
  misc_feature 1..22: note = Synthetic DNA
  source 1..22: mol_type = other DNA
cggagcctcacgcgatgatcta

SEQ ID NO: 36 - DNA, 29 bp, synthetic construct
  misc_feature 1..29: note = Synthetic DNA
  source 1..29: mol_type = other DNA
agtacactgtagttgtcctcagatactcc

SEQ ID NO: 37 - DNA, 26 bp, synthetic construct
  misc_feature 1..26: note = Synthetic DNA
  source 1..26: mol_type = other DNA
tccaccccaaacatttccactaactg

SEQ ID NO: 38 - DNA, 20 bp, synthetic construct
  misc_feature 1..20: note = Synthetic DNA
  source 1..20: mol_type = other DNA
tgccaggccaggatctgctg

SEQ ID NO: 39 - DNA, 20 bp, synthetic construct
  misc_feature 1..20: note = Synthetic DNA
  source 1..20: mol_type = other DNA
atccggtgcttggcttgatg

SEQ ID NO: 40 - DNA, 22 bp, synthetic construct
  misc_feature 1..22: note = Synthetic DNA
  source 1..22: mol_type = other DNA
cacatgtcccttctgccataag

SEQ ID NO: 41 - DNA, 21 bp, synthetic construct
  misc_feature 1..21: note = Synthetic DNA
  source 1..21: mol_type = other DNA
agagatcactgaagctgctac

SEQ ID NO: 42 - DNA, 22 bp, synthetic construct
  misc_feature 1..22: note = Synthetic DNA
  source 1..22: mol_type = other DNA
tctagtcccttcaagggctgag

SEQ ID NO: 43 - DNA, 24 bp, synthetic construct
  misc_feature 1..24: note = Synthetic DNA
  source 1..24: mol_type = other DNA
acaatgtctctctgaaggctgtac

SEQ ID NO: 44 - DNA, 20 bp, synthetic construct
  misc_feature 1..20: note = Synthetic DNA
  source 1..20: mol_type = other DNA
aacatcaccgtgacatgcag

SEQ ID NO: 45 - DNA, 21 bp, synthetic construct
  misc_feature 1..21: note = Synthetic DNA
  source 1..21: mol_type = other DNA
tgtctgccaatgactctgaag

SEQ ID NO: 46 - DNA, 23 bp, synthetic construct
  misc_feature 1..23: note = Synthetic DNA
  source 1..23: mol_type = other DNA
cagctgcagcaattaccggagtg

SEQ ID NO: 47 - DNA, 23 bp, synthetic construct
  misc_feature 1..23: note = Synthetic DNA
  source 1..23: mol_type = other DNA
gaagggaggcatgtcagtaggtc

SEQ ID NO: 48 - DNA, 20 bp, synthetic construct
  misc_feature 1..20: note = Synthetic DNA
  source 1..20: mol_type = other DNA
cctttgtgacagcgcacgtt

SEQ ID NO: 49 - DNA, 20 bp, synthetic construct
  misc_feature 1..20: note = Synthetic DNA
  source 1..20: mol_type = other DNA
ccagacactagggctttcgt

SEQ ID NO: 50 - DNA, 23 bp, synthetic construct
  misc_feature 1..23: note = Synthetic DNA
  source 1..23: mol_type = other DNA
cggctggatgaggtcatctccaa

SEQ ID NO: 51 - DNA, 22 bp, synthetic construct
  misc_feature 1..22: note = Synthetic DNA
  source 1..22: mol_type = other DNA
gactcaactctgggagctcatg

SEQ ID NO: 52 - DNA, 22 bp, synthetic construct
  misc_feature 1..22: note = Synthetic DNA
  source 1..22: mol_type = other DNA
gtttcaaacaggtggctcatgc

SEQ ID NO: 53 - DNA, 20 bp, synthetic construct
  source 1..20: mol_type = other DNA
atgctgtactgccatacgaa

SEQ ID NO: 54 - DNA, 20 bp, synthetic construct
  source 1..20: mol_type = other DNA
gatgtatccactcacgcact

SEQ ID NO: 55 - DNA, 20 bp, synthetic construct
  source 1..20: mol_type = other DNA
attaaggacactaatacctg

SEQ ID NO: 56 - DNA, 20 bp, synthetic construct
  source 1..20: mol_type = other DNA
cacacattgctgatctgctg

SEQ ID NO: 57 - DNA, 20 bp, synthetic construct
  source 1..20: mol_type = other DNA
aatatgattggattgtacgt

SEQ ID NO: 58 - DNA, 20 bp, synthetic construct
  source 1..20: mol_type = other DNA
catcaatgcatagatgtctg

SEQ ID NO: 59 - DNA, 20 bp, synthetic construct
  source 1..20: mol_type = other DNA
tcatctggggaagtgcatcg

SEQ ID NO: 60 - DNA, 20 bp, synthetic construct
  source 1..20: mol_type = other DNA
aagactggagttgtgtccac

SEQ ID NO: 61 - DNA, 20 bp, synthetic construct
  source 1..20: mol_type = other DNA
gatgctctgttgaaacgtga

SEQ ID NO: 62 - DNA, 20 bp, synthetic construct
  source 1..20: mol_type = other DNA
ccaagcaatctgacctgctg

SEQ ID NO: 63 - DNA, 20 bp, synthetic construct
  source 1..20: mol_type = other DNA
catgagaagcacgcatacga

SEQ ID NO: 64 - DNA, 20 bp, synthetic construct
  source 1..20: mol_type = other DNA
ctgagatcacccgtagagag

SEQ ID NO: 65 - DNA, 20 bp, synthetic construct
  source 1..20: mol_type = other DNA
cttcatccttctgccaggtc

SEQ ID NO: 66 - DNA, 20 bp, synthetic construct
  source 1..20: mol_type = other DNA
gctgacagctctggttcggt

SEQ ID NO: 67 - DNA, 20 bp, synthetic construct
  source 1..20: mol_type = other DNA
tctgctgtgatgggtcacat

SEQ ID NO: 68 - DNA, 21 bp, synthetic construct
  source 1..21: mol_type = other DNA
tctgatggaggtcagccagac

SEQ ID NO: 69 - DNA, 22 bp, synthetic construct
  source 1..22: mol_type = other DNA
tgtgtttcctactgcaaggatc

SEQ ID NO: 70 - DNA, 21 bp, synthetic construct
  source 1..21: mol_type = other DNA
tgacgccatgcttcggctagc

SEQ ID NO: 71 - DNA, 22 bp, synthetic construct
  source 1..22: mol_type = other DNA
cagacccagtttgagtcagtag

SEQ ID NO: 72 - DNA, 20 bp, synthetic construct
  source 1..20: mol_type = other DNA
aagagcttaaggctgctctg

SEQ ID NO: 73 - DNA, 20 bp, synthetic construct
  source 1..20: mol_type = other DNA
ccaggagatgtctcaatgct

SEQ ID NO: 74 - DNA, 27 bp, synthetic construct
  source 1..27: mol_type = other DNA
tcatcacataatgtaaagatacctgtg

SEQ ID NO: 75 - DNA, 20 bp, synthetic construct
  source 1..20: mol_type = other DNA
gtggagtcacccatgtgctt

SEQ ID NO: 76 - DNA, 23 bp, synthetic construct
  source 1..23: mol_type = other DNA
atttgtagcctcacattcaatgc

SEQ ID NO: 77 - DNA, 25 bp, synthetic construct
  source 1..25: mol_type = other DNA
ggctgttgacttcccaactctaatc

SEQ ID NO: 78 - DNA, 25 bp, synthetic construct
  source 1..25: mol_type = other DNA
tgctcaccggagctttggccttgac

SEQ ID NO: 79 - DNA, 25 bp, synthetic construct
  source 1..25: mol_type = other DNA
actgaagcaatgtttatggaccatc

SEQ ID NO: 80 - DNA, 20 bp, synthetic construct
  source 1..20: mol_type = other DNA
caagatggacttcgggactc

SEQ ID NO: 81 - DNA, 20 bp, synthetic construct
  source 1..20: mol_type = other DNA
ccttccaggatcatacagcc

SEQ ID NO: 82 - DNA, 20 bp, synthetic construct
  source 1..20: mol_type = other DNA
ctccacaagctccatgtcct

SEQ ID NO: 83 - DNA, 20 bp, synthetic construct
  source 1..20: mol_type = other DNA
tggatccagactcccgtatg

SEQ ID NO: 84 - DNA, 20 bp, synthetic construct
  source 1..20: mol_type = other DNA
gtgagagtcatgatgcccag

SEQ ID NO: 85 - DNA, 20 bp, synthetic construct
  source 1..20: mol_type = other DNA
ggaggatgaaagggctaagc

SEQ ID NO: 86 - DNA, 21 bp, synthetic construct
  source 1..21: mol_type = other DNA
ctcaggagacatgagctccag

SEQ ID NO: 87 - DNA, 20 bp, synthetic construct
  source 1..20: mol_type = other DNA
tttggagacttcgcccactc

SEQ ID NO: 88 - DNA, 20 bp, synthetic construct
  source 1..20: mol_type = other DNA
actctgggaggcactaggag

SEQ ID NO: 89 - DNA, 20 bp, synthetic construct
  source 1..20: mol_type = other DNA
caatggctcatgtggattcc

SEQ ID NO: 90 - DNA, 20 bp, synthetic construct
  source 1..20: mol_type = other DNA
cttccttaccccatttcagg

SEQ ID NO: 91 - DNA, 21 bp, synthetic construct
  source 1..21: mol_type = other DNA
ctacttcacgcataccgtcag

SEQ ID NO: 92 - DNA, 20 bp, synthetic construct
  source 1..20: mol_type = other DNA
cacctgcagaaacgttctgg

SEQ ID NO: 93 - DNA, 25 bp, synthetic construct
  source 1..25: mol_type = other DNA
atcattcctaggctgcatcactcag

SEQ ID NO: 94 - DNA, 25 bp, synthetic construct
  source 1..25: mol_type = other DNA
cctcactcatggaggaggctgatgc

SEQ ID NO: 95 - DNA, 20 bp, synthetic construct
  source 1..20: mol_type = other DNA
ttcactttctgggaagtacg

SEQ ID NO: 96 - DNA, 25 bp, synthetic construct
  source 1..25: mol_type = other DNA
gaccgtaggaccatttgccatgttc

SEQ ID NO: 97 - DNA, 25 bp, synthetic construct
  source 1..25: mol_type = other DNA
tcactgataccaagcagtagttctg

SEQ ID NO: 98 - DNA, 24 bp, synthetic construct
  source 1..24: mol_type = other DNA
acacttgaagttattgtcatacag

SEQ ID NO: 99 - DNA, 23 bp, synthetic construct
  source 1..23: mol_type = other DNA
atttgtagcctcacattcaatgc

SEQ ID NO: 100 - DNA, 25 bp, synthetic construct
  source 1..25: mol_type = other DNA
ggctgttgacttcccaactctaatc

SEQ ID NO: 101 - DNA, 20 bp, synthetic construct
  source 1..20: mol_type = other DNA
agcacagctcctgacttctg